European Patent Specification EP 3 786 284 B1, published August 6, 2025. Title: Scaffold including multi-layer graphene film for promoting of stem cell differentiation. Applicant: Seoul National University R&DB Foundation. The sequence listing filed with the application follows.

SEQUENCE LISTING (6 sequences)

SEQ ID NO: 1 - DNA, 19 bp, Artificial Sequence
  RUNX2 forward primer
gacagccccaacttcctgt

SEQ ID NO: 2 - DNA, 20 bp, Artificial Sequence
  RUNX2 reverse primer
ccggagctcagcagaataat

SEQ ID NO: 3 - DNA, 20 bp, Artificial Sequence
  OSTEOCALCIN forward primer
agcaaaggtgcagcctttgt

SEQ ID NO: 4 - DNA, 19 bp, Artificial Sequence
  OSTEOCALCIN reverse primer
gcgcctgggtctcttcact

SEQ ID NO: 5 - DNA, 20 bp, Artificial Sequence
  GAPDH forward primer
gagtcaacggatttggtcgt

SEQ ID NO: 6 - DNA, 20 bp, Artificial Sequence
  GAPDH reverse primer
ttgattttggagggatctcg